European Patent Specification EP 3 458 601 B1, published July 5, 2023. Title: METHODS FOR DETECTING TARGET NUCLEIC ACIDS IN A SAMPLE. Applicant: NanoString Technologies, Inc. KHAFIZOV, Rustem DUNAWAY, Dwayne GREGORY, Mark. The sequence listing filed with the application follows.

SEQUENCE LISTING (102 sequences)

SEQ ID NO: 1 - DNA, 10 bp, Artificial Sequence
  Synthetic Polynucleotide
atacatctag

SEQ ID NO: 2 - DNA, 10 bp, Artificial Sequence
  Synthetic Polynucleotide
gatctacata

SEQ ID NO: 3 - DNA, 10 bp, Artificial Sequence
  Synthetic Polynucleotide
ttaggtaaag

SEQ ID NO: 4 - DNA, 10 bp, Artificial Sequence
  Synthetic Polynucleotide
tcttcattac

SEQ ID NO: 5 - DNA, 10 bp, Artificial Sequence
  Synthetic Polynucleotide
atgaatctac

SEQ ID NO: 6 - DNA, 10 bp, Artificial Sequence
  Synthetic Polynucleotide
tcaatgtatg

SEQ ID NO: 7 - DNA, 10 bp, Artificial Sequence
  Synthetic Polynucleotide
aattgagtac

SEQ ID NO: 8 - DNA, 10 bp, Artificial Sequence
  Synthetic Polynucleotide
atgttaatgg

SEQ ID NO: 9 - DNA, 10 bp, Artificial Sequence
  Synthetic Polynucleotide
aattaggatg

SEQ ID NO: 10 - DNA, 10 bp, Artificial Sequence
  Synthetic Polynucleotide
ataatggatc

SEQ ID NO: 11 - DNA, 10 bp, Artificial Sequence
  Synthetic Polynucleotide
taataaggtg

SEQ ID NO: 12 - DNA, 10 bp, Artificial Sequence
  Synthetic Polynucleotide
tagttagagc

SEQ ID NO: 13 - DNA, 10 bp, Artificial Sequence
  Synthetic Polynucleotide
atagagaagg

SEQ ID NO: 14 - DNA, 10 bp, Artificial Sequence
  Synthetic Polynucleotide
ttgatgatac

SEQ ID NO: 15 - DNA, 10 bp, Artificial Sequence
  Synthetic Polynucleotide
atagtgattc

SEQ ID NO: 16 - DNA, 10 bp, Artificial Sequence
  Synthetic Polynucleotide
tataacgatg

SEQ ID NO: 17 - DNA, 10 bp, Artificial Sequence
  Synthetic Polynucleotide
ttaagtttag

SEQ ID NO: 18 - DNA, 10 bp, Artificial Sequence
  Synthetic Polynucleotide
atacgttatg

SEQ ID NO: 19 - DNA, 10 bp, Artificial Sequence
  Synthetic Polynucleotide
tgtactatag

SEQ ID NO: 20 - DNA, 10 bp, Artificial Sequence
  Synthetic Polynucleotide
ttaacaagtg

SEQ ID NO: 21 - DNA, 10 bp, Artificial Sequence
  Synthetic Polynucleotide
aactatgtac

SEQ ID NO: 22 - DNA, 10 bp, Artificial Sequence
  Synthetic Polynucleotide
taactatgac

SEQ ID NO: 23 - DNA, 10 bp, Artificial Sequence
  Synthetic Polynucleotide
actaatgttc

SEQ ID NO: 24 - DNA, 10 bp, Artificial Sequence
  Synthetic Polynucleotide
tcattgaatg

SEQ ID NO: 25 - DNA, 14 bp, Artificial Sequence
  Synthetic Polynucleotide
ctgtctcatctctt

SEQ ID NO: 26 - DNA, 26 bp, Artificial Sequence
  Synthetic Polynucleotide
ctgtctcatctcttgctgcatcctgt

SEQ ID NO: 27 - DNA, 38 bp, Artificial Sequence
  Synthetic Polynucleotide
ctgtctcatctcttgctgcatcctgtcggttcacgttg

SEQ ID NO: 28 - DNA, 36 bp, Artificial Sequence
  Synthetic Polynucleotide
ctgtctcatcttgctgcatcctgtcggttcacgttg

SEQ ID NO: 29 - DNA, 36 bp, Artificial Sequence
  Synthetic Polynucleotide
ctgtctcattttgctgcatcctgtccgttcacgttg

SEQ ID NO: 30 - DNA, 12 bp, Artificial Sequence
  Synthetic Polynucleotide
cacgaacgtcag

SEQ ID NO: 31 - DNA, 12 bp, Artificial Sequence
  Synthetic Polynucleotide
catcgcatgcct

SEQ ID NO: 32 - DNA, 12 bp, Artificial Sequence
  Synthetic Polynucleotide
gtcatctcctac

SEQ ID NO: 33 - DNA, 12 bp, Artificial Sequence
  Synthetic Polynucleotide
gtcatccgctac

SEQ ID NO: 34 - DNA, 12 bp, Artificial Sequence
  Synthetic Polynucleotide
gtcatcgactac

SEQ ID NO: 35 - DNA, 12 bp, Artificial Sequence
  Synthetic Polynucleotide
gtcatcttctac

SEQ ID NO: 36 - DNA, 12 bp, Artificial Sequence
  Synthetic Polynucleotide
gtcatcacctac

SEQ ID NO: 37 - DNA, 12 bp, Artificial Sequence
  Synthetic Polynucleotide
gtcatcactcac

SEQ ID NO: 38 - DNA, 12 bp, Artificial Sequence
  Synthetic Polynucleotide
gtcatcttcgac

SEQ ID NO: 39 - DNA, 12 bp, Artificial Sequence
  Synthetic Polynucleotide
gtcatcaactac

SEQ ID NO: 40 - DNA, 12 bp, Artificial Sequence
  Synthetic Polynucleotide
gtcatccgtaac

SEQ ID NO: 41 - DNA, 12 bp, Artificial Sequence
  Synthetic Polynucleotide
gtcatccgaaac

SEQ ID NO: 42 - DNA, 12 bp, Artificial Sequence
  Synthetic Polynucleotide
gtcatcacaaac

SEQ ID NO: 43 - DNA, 12 bp, Artificial Sequence
  Synthetic Polynucleotide
gtcatcttgcac

SEQ ID NO: 44 - DNA, 12 bp, Artificial Sequence
  Synthetic Polynucleotide
gtcatcttgcct

SEQ ID NO: 45 - DNA, 12 bp, Artificial Sequence
  Synthetic Polynucleotide
gtcatccgtcct

SEQ ID NO: 46 - DNA, 12 bp, Artificial Sequence
  Synthetic Polynucleotide
cttttcacctct

SEQ ID NO: 47 - DNA, 12 bp, Artificial Sequence
  Synthetic Polynucleotide
cttttcctctct

SEQ ID NO: 48 - DNA, 12 bp, Artificial Sequence
  Synthetic Polynucleotide
cttttcgactct

SEQ ID NO: 49 - DNA, 12 bp, Artificial Sequence
  Synthetic Polynucleotide
cttttctgctct

SEQ ID NO: 50 - DNA, 12 bp, Artificial Sequence
  Synthetic Polynucleotide
cttttctgtact

SEQ ID NO: 51 - DNA, 12 bp, Artificial Sequence
  Synthetic Polynucleotide
cttttctgtgct

SEQ ID NO: 52 - DNA, 12 bp, Artificial Sequence
  Synthetic Polynucleotide
cttttctgtcct

SEQ ID NO: 53 - DNA, 12 bp, Artificial Sequence
  Synthetic Polynucleotide
cttttcactcct

SEQ ID NO: 54 - DNA, 12 bp, Artificial Sequence
  Synthetic Polynucleotide
cttttcgttcct

SEQ ID NO: 55 - DNA, 12 bp, Artificial Sequence
  Synthetic Polynucleotide
cttttcgtacct

SEQ ID NO: 56 - DNA, 12 bp, Artificial Sequence
  Synthetic Polynucleotide
cttttccgtcct

SEQ ID NO: 57 - DNA, 12 bp, Artificial Sequence
  Synthetic Polynucleotide
cttttctgacct

SEQ ID NO: 58 - DNA, 12 bp, Artificial Sequence
  Synthetic Polynucleotide
aggcatgcgatg

SEQ ID NO: 59 - DNA, 12 bp, Artificial Sequence
  Synthetic Polynucleotide
aggcattgtgct

SEQ ID NO: 60 - DNA, 12 bp, Artificial Sequence
  Synthetic Polynucleotide
aggcattgctct

SEQ ID NO: 61 - DNA, 12 bp, Artificial Sequence
  Synthetic Polynucleotide
aggcatttctac

SEQ ID NO: 62 - DNA, 12 bp, Artificial Sequence
  Synthetic Polynucleotide
aggcatacctac

SEQ ID NO: 63 - DNA, 12 bp, Artificial Sequence
  Synthetic Polynucleotide
aggcatttgcac

SEQ ID NO: 64 - DNA, 12 bp, Artificial Sequence
  Synthetic Polynucleotide
aggcatcgtcct

SEQ ID NO: 65 - DNA, 12 bp, Artificial Sequence
  Synthetic Polynucleotide
tcctgtcggttc

SEQ ID NO: 66 - DNA, 12 bp, Artificial Sequence
  Synthetic Polynucleotide
gttcaatgctct

SEQ ID NO: 67 - DNA, 12 bp, Artificial Sequence
  Synthetic Polynucleotide
attcggtgctct

SEQ ID NO: 68 - DNA, 12 bp, Artificial Sequence
  Synthetic Polynucleotide
gatgcctgctct

SEQ ID NO: 69 - DNA, 12 bp, Artificial Sequence
  Synthetic Polynucleotide
tttgcttgctct

SEQ ID NO: 70 - DNA, 100 bp, Artificial Sequence
  Synthetic Polynucleotide
ttcactgtagctgtctcattttgctgcatcctgtccgttcacgttggagcttgtcatccgtcctcttttcactcctaggcatttgcctattcggcgtcct

SEQ ID NO: 71 - DNA, 15 bp, Artificial Sequence
  Synthetic Construct
  misc_feature: /5Alex488N/
cctgcgaatgagtcg

SEQ ID NO: 72 - DNA, 15 bp, Artificial Sequence
  Synthetic Construct
  misc_feature: /5Alex546N/
tcgagtgcatgagct

SEQ ID NO: 73 - DNA, 15 bp, Artificial Sequence
  Synthetic Construct
  misc_feature: /5Alex647N/
agtagacctggcgtc

SEQ ID NO: 74 - DNA, 15 bp, Artificial Sequence
  Synthetic Construct
  misc_feature: /5TexRd-XN/
atcaccgtgcagcta

SEQ ID NO: 75 - DNA, 89 bp, Artificial Sequence
  Synthetic Construct
tgcgacgcacctatcgactcattcgcaggcgactcattcgcaggcgactcattcgcaggcgactcattcgcaggcgactcattcgcagg

SEQ ID NO: 76 - DNA, 89 bp, Artificial Sequence
  Synthetic Construct
aaggtgtgcagcctagctcatgcactcgaagctcatgcactcgaagctcatgcactcgaagctcatgcactcgaagctcatgcactcga

SEQ ID NO: 77 - DNA, 89 bp, Artificial Sequence
  Synthetic Construct
actgttgccgccaagacgccaggtctactgacgccaggtctactgacgccaggtctactgacgccaggtctactgacgccaggtctact

SEQ ID NO: 78 - DNA, 89 bp, Artificial Sequence
  Synthetic Construct
aacgccatttgccgtagctgcacggtgattagctgcacggtgattagctgcacggtgattagctgcacggtgattagctgcacggtgat

SEQ ID NO: 79 - DNA, 96 bp, Artificial Sequence
  Synthetic Construct
aggctgcacaccttaggctgcacaccttaggctgcacaccttaggctgcacaccttaggctgcacaccttaggctgcacaccttaggcgagatgac

SEQ ID NO: 80 - DNA, 96 bp, Artificial Sequence
  Synthetic Construct
aggctgcacaccttaggctgcacaccttaggctgcacaccttcggcaaatggcgttcggcaaatggcgttcggcaaatggcgttagggaagatgac

SEQ ID NO: 81 - DNA, 96 bp, Artificial Sequence
  Synthetic Construct
cggcaaatggcgttcggcaaatggcgttcggcaaatggcgttcggcaaatggcgttcggcaaatggcgttcggcaaatggcgttagggtggatgac

SEQ ID NO: 82 - DNA, 96 bp, Artificial Sequence
  Synthetic Construct
ataggtgcgtcgcaataggtgcgtcgcaataggtgcgtcgcaataggtgcgtcgcaataggtgcgtcgcaataggtgcgtcgcaaggacagatgac

SEQ ID NO: 83 - DNA, 96 bp, Artificial Sequence
  Synthetic Construct
ttggcggcaacagtttggcggcaacagtttggcggcaacagtttggcggcaacagtttggcggcaacagtttggcggcaacagtaggttagatgac

SEQ ID NO: 84 - DNA, 96 bp, Artificial Sequence
  Synthetic Construct
aggctgcacaccttaggctgcacaccttaggctgcacaccttttggcggcaacagtttggcggcaacagtttggcggcaacagtgtagaagatgac

SEQ ID NO: 85 - DNA, 96 bp, Artificial Sequence
  Synthetic Construct
cggcaaatggcgttcggcaaatggcgttcggcaaatggcgttttggcggcaacagtttggcggcaacagtttggcggcaacagtaggaacgatgac

SEQ ID NO: 86 - DNA, 96 bp, Artificial Sequence
  Synthetic Construct
ataggtgcgtcgcaataggtgcgtcgcaataggtgcgtcgcattggcggcaacagtttggcggcaacagtttggcggcaacagtaggagtgatgac

SEQ ID NO: 87 - DNA, 96 bp, Artificial Sequence
  Synthetic Construct
ataggtgcgtcgcaataggtgcgtcgcaataggtgcgtcgcaataggtgcgtcgcaataggtgcgtcgcaataggtgcgtcgcaagccatgaaaag

SEQ ID NO: 88 - DNA, 96 bp, Artificial Sequence
  Synthetic Construct
ataggtgcgtcgcaataggtgcgtcgcaataggtgcgtcgcaaggctgcacaccttaggctgcacaccttaggctgcacaccttagcgctgaaaag

SEQ ID NO: 89 - DNA, 96 bp, Artificial Sequence
  Synthetic Construct
ataggtgcgtcgcaataggtgcgtcgcaataggtgcgtcgcacggcaaatggcgttcggcaaatggcgttcggcaaatggcgttagcatcgaaaag

SEQ ID NO: 90 - DNA, 96 bp, Artificial Sequence
  Synthetic Construct
aggctgcacaccttaggctgcacaccttaggctgcacaccttaggctgcacaccttaggctgcacaccttaggctgcacaccttagccgagaaaag

SEQ ID NO: 91 - DNA, 96 bp, Artificial Sequence
  Synthetic Construct
aggctgcacaccttaggctgcacaccttaggctgcacaccttttggcggcaacagtttggcggcaacagtttggcggcaacagtagctgggaaaag

SEQ ID NO: 92 - DNA, 96 bp, Artificial Sequence
  Synthetic Construct
aggctgcacaccttaggctgcacaccttaggctgcacaccttcggcaaatggcgttcggcaaatggcgttcggcaaatggcgttagcgaagaaaag

SEQ ID NO: 93 - DNA, 96 bp, Artificial Sequence
  Synthetic Construct
ttggcggcaacagtttggcggcaacagtttggcggcaacagtttggcggcaacagtttggcggcaacagtttggcggcaacagtagctcggaaaag

SEQ ID NO: 94 - DNA, 96 bp, Artificial Sequence
  Synthetic Construct
cggcaaatggcgttcggcaaatggcgttcggcaaatggcgttcggcaaatggcgttcggcaaatggcgttcggcaaatggcgttagcgtggaaaag

SEQ ID NO: 95 - DNA, 96 bp, Artificial Sequence
  Synthetic Construct
ataggtgcgtcgcaataggtgcgtcgcaataggtgcgtcgcaaggctgcacaccttaggctgcacaccttaggctgcacaccttgtaagtccgaat

SEQ ID NO: 96 - DNA, 96 bp, Artificial Sequence
  Synthetic Construct
cggcaaatggcgttcggcaaatggcgttcggcaaatggcgttttggcggcaacagtttggcggcaacagtttggcggcaacagtgtaacaccgaat

SEQ ID NO: 97 - DNA, 96 bp, Artificial Sequence
  Synthetic Construct
ataggtgcgtcgcaataggtgcgtcgcaataggtgcgtcgcaataggtgcgtcgcaataggtgcgtcgcaataggtgcgtcgcagtacatccgaat

SEQ ID NO: 98 - DNA, 96 bp, Artificial Sequence
  Synthetic Construct
ataggtgcgtcgcaataggtgcgtcgcaataggtgcgtcgcacggcaaatggcgttcggcaaatggcgttcggcaaatggcgttgtaatcccgaat

SEQ ID NO: 99 - DNA, 96 bp, Artificial Sequence
  Synthetic Construct
aggctgcacaccttaggctgcacaccttaggctgcacaccttaggctgcacaccttaggctgcacaccttaggctgcacaccttgtacgaccgaat

SEQ ID NO: 100 - DNA, 96 bp, Artificial Sequence
  Synthetic Construct
aggctgcacaccttaggctgcacaccttaggctgcacaccttcggcaaatggcgttcggcaaatggcgttcggcaaatggcgttgtagaaccgaat

SEQ ID NO: 101 - DNA, 96 bp, Artificial Sequence
  Synthetic Construct
ttggcggcaacagtttggcggcaacagtttggcggcaacagtttggcggcaacagtttggcggcaacagtttggcggcaacagtgtatcgccgaat

SEQ ID NO: 102 - DNA, 96 bp, Artificial Sequence
  Synthetic Construct
aggctgcacaccttaggctgcacaccttaggctgcacaccttttggcggcaacagtttggcggcaacagtttggcggcaacagtgtagttccgaat